European Patent Specification EP 4 536 686 B1, published November 19, 2025. Title: PEPTIDE-MODIFIED AAV CAPSID WITH ENHANCED MUSCLE TRANSDUCTION EFFICIENCY. Applicant: GENETHON. The sequence listing filed with the application follows.

SEQUENCE LISTING (46 sequences)

SEQ ID NO: 1 - protein, 7 aa, synthetic construct
  REGION 1..7: note = synthetic peptide (ITGAV-B6 binding motif)
  VARIANT 5..6: note = XaXa is any pair of amino acid except GS and ST
  VARIANT 7: note = Xa is L or I
RGDLXXX

SEQ ID NO: 2 - protein, 7 aa, synthetic construct
  REGION 1..7: note = synthetic peptide (4um9 (4um9_native))
RGDLGRL

SEQ ID NO: 3 - protein, 7 aa, synthetic construct
  REGION 1..7: note = synthetic peptide (4um9_modified)
RGDLGEL

SEQ ID NO: 4 - protein, 7 aa, synthetic construct
  REGION 1..7: note = synthetic peptide (5off)
RGDLATI

SEQ ID NO: 5 - protein, 7 aa, synthetic construct
  REGION 1..7: note = synthetic peptide (5off_modified)
RGDLAEL

SEQ ID NO: 6 - protein, 7 aa, synthetic construct
  REGION 1..7: note = synthetic peptide (5nem)
RGDLQVL

SEQ ID NO: 7 - protein, 7 aa, synthetic construct
  REGION 1..7: note = synthetic peptide (5nem_modified)
RGDLAEI

SEQ ID NO: 8 - protein, 8 aa, synthetic construct
  REGION 1..8: note = synthetic peptide (4um9 + G)
GRGDLGRL

SEQ ID NO: 9 - protein, 8 aa, synthetic construct
  REGION 1..8: note = synthetic peptide (4um9_modified + P)
PRGDLGEL

SEQ ID NO: 10 - protein, 8 aa, synthetic construct
  REGION 1..8: note = synthetic peptide (5off + R)
RRGDLATI

SEQ ID NO: 11 - protein, 8 aa, synthetic construct
  REGION 1..8: note = synthetic peptide (5off_modified + Q)
QRGDLAEL

SEQ ID NO: 12 - protein, 8 aa, synthetic construct
  REGION 1..8: note = synthetic peptide (5nem + V)
VRGDLQVL

SEQ ID NO: 13 - protein, 8 aa, synthetic construct
  REGION 1..8: note = synthetic peptide (5nem_modified + V)
VRGDLAEI

SEQ ID NO: 14 - protein, 12 aa, synthetic construct
  REGION 1..12: note = synthetic peptide (4um9 + linker)
TDGRGDLGRLGP

SEQ ID NO: 15 - protein, 12 aa, synthetic construct
  REGION 1..12: note = synthetic peptide (4um9_modified + linker)
SEPRGDLGELNA

SEQ ID NO: 16 - protein, 12 aa, synthetic construct
  REGION 1..12: note = synthetic peptide (5off + linker)
EPRRGDLATIGS

SEQ ID NO: 17 - protein, 12 aa, synthetic construct
  REGION 1..12: note = synthetic peptide (5off_modified + linker)
TDQRGDLAELHG

SEQ ID NO: 18 - protein, 12 aa, synthetic construct
  REGION 1..12: note = synthetic peptide (5nem + linker)
APVRGDLQVLAP

SEQ ID NO: 19 - protein, 12 aa, synthetic construct
  REGION 1..12: note = synthetic peptide (5nem_modified + linker)
APVRGDLAEINP

SEQ ID NO: 20 - protein, 737 aa, synthetic construct
  REGION 1..737: note = synthetic polypeptide (AAV9.rh74 capsid (VP1 protein))
MAADGYLPDWLEDNLSEGIREWWALKPGAPQPKANQQHQDNARGLVLPGYKYLGPGNGLDKGEPVNAADAAALEHDKAYDQQLKAGDNPYLKYNHADAEFQERLKEDTSFGGNLGRAVFQAKKRLLEPLGLVEEAAKTAPGKKRPVEQSPQEPDSSAGIGKSGAQPAKKRLNFGQTGDTESVPDPQPIGEPPAAPSGVGSLTMASGGGAPVADNNEGADGVGSSSGNWHCDSQWLGDRVITTSTRTWALPTYNNHLYKQISNSTSGGSSNDNAYFGYSTPWGYFDFNRFHCHFSPRDWQRLINNNWGFRPKRLNFKLFNIQVKEVTDNNGVKTIANNLTSTVQVFTDSDYQLPYVLGSAHEGCLPPFPADVFMIPQYGYLTLNDGSQAVGRSSFYCLEYFPSQMLRTGNNFQFSYEFENVPFHSSYAHSQSLDRLMNPLIDQYLYYLSRTQSTGGTAGTQQLLFSQAGPNNMSAQAKNWLPGPCYRQQRVSTTLSQNNNSNFAWTGATKYHLNGRDSLVNPGVAMATHKDDEERFFPSSGVLMFGKQGAGKDNVDYSSVMLTSEEEIKTTNPVATEQYGVVADNLQQQNAAPIVGAVNSQGALPGMVWQNRDVYLQGPIWAKIPHTDGNFHPSPLMGGFGMKHPPPQILIKNTPVPADPPTAFNKDKLNSFITQYSTGQVSVEIEWELQKENSKRWNPEIQYTSNYYKSNNVEFAVNTEGVYSEPRPIGTRYLTRNL

SEQ ID NO: 21 - protein, 742 aa, synthetic construct
  REGION 1..742: note = synthetic polypeptide (Cap9rh74_VR4-4um9 (LICA.01) (VP1 protein))
MAADGYLPDWLEDNLSEGIREWWALKPGAPQPKANQQHQDNARGLVLPGYKYLGPGNGLDKGEPVNAADAAALEHDKAYDQQLKAGDNPYLKYNHADAEFQERLKEDTSFGGNLGRAVFQAKKRLLEPLGLVEEAAKTAPGKKRPVEQSPQEPDSSAGIGKSGAQPAKKRLNFGQTGDTESVPDPQPIGEPPAAPSGVGSLTMASGGGAPVADNNEGADGVGSSSGNWHCDSQWLGDRVITTSTRTWALPTYNNHLYKQISNSTSGGSSNDNAYFGYSTPWGYFDFNRFHCHFSPRDWQRLINNNWGFRPKRLNFKLFNIQVKEVTDNNGVKTIANNLTSTVQVFTDSDYQLPYVLGSAHEGCLPPFPADVFMIPQYGYLTLNDGSQAVGRSSFYCLEYFPSQMLRTGNNFQFSYEFENVPFHSSYAHSQSLDRLMNPLIDQYLYYLSRTQSTDGRGDLGRLGPQQLLFSQAGPNNMSAQAKNWLPGPCYRQQRVSTTLSQNNNSNFAWTGATKYHLNGRDSLVNPGVAMATHKDDEERFFPSSGVLMFGKQGAGKDNVDYSSVMLTSEEEIKTTNPVATEQYGVVADNLQQQNAAPIVGAVNSQGALPGMVWQNRDVYLQGPIWAKIPHTDGNFHPSPLMGGFGMKHPPPQILIKNTPVPADPPTAFNKDKLNSFITQYSTGQVSVEIEWELQKENSKRWNPEIQYTSNYYKSNNVEFAVNTEGVYSEPRPIGTRYLTRNL

SEQ ID NO: 22 - protein, 742 aa, synthetic construct
  REGION 1..742: note = synthetic polypeptide (Cap9rh74_VR4-4um9_modified (VP1 protein))
MAADGYLPDWLEDNLSEGIREWWALKPGAPQPKANQQHQDNARGLVLPGYKYLGPGNGLDKGEPVNAADAAALEHDKAYDQQLKAGDNPYLKYNHADAEFQERLKEDTSFGGNLGRAVFQAKKRLLEPLGLVEEAAKTAPGKKRPVEQSPQEPDSSAGIGKSGAQPAKKRLNFGQTGDTESVPDPQPIGEPPAAPSGVGSLTMASGGGAPVADNNEGADGVGSSSGNWHCDSQWLGDRVITTSTRTWALPTYNNHLYKQISNSTSGGSSNDNAYFGYSTPWGYFDFNRFHCHFSPRDWQRLINNNWGFRPKRLNFKLFNIQVKEVTDNNGVKTIANNLTSTVQVFTDSDYQLPYVLGSAHEGCLPPFPADVFMIPQYGYLTLNDGSQAVGRSSFYCLEYFPSQMLRTGNNFQFSYEFENVPFHSSYAHSQSLDRLMNPLIDQYLYYLSRTQSSEPRGDLGELNAQQLLFSQAGPNNMSAQAKNWLPGPCYRQQRVSTTLSQNNNSNFAWTGATKYHLNGRDSLVNPGVAMATHKDDEERFFPSSGVLMFGKQGAGKDNVDYSSVMLTSEEEIKTTNPVATEQYGVVADNLQQQNAAPIVGAVNSQGALPGMVWQNRDVYLQGPIWAKIPHTDGNFHPSPLMGGFGMKHPPPQILIKNTPVPADPPTAFNKDKLNSFITQYSTGQVSVEIEWELQKENSKRWNPEIQYTSNYYKSNNVEFAVNTEGVYSEPRPIGTRYLTRNL

SEQ ID NO: 23 - protein, 742 aa, synthetic construct
  REGION 1..742: note = synthetic polypeptide (Cap9rh74_VR4-5ffo (VP1 protein))
MAADGYLPDWLEDNLSEGIREWWALKPGAPQPKANQQHQDNARGLVLPGYKYLGPGNGLDKGEPVNAADAAALEHDKAYDQQLKAGDNPYLKYNHADAEFQERLKEDTSFGGNLGRAVFQAKKRLLEPLGLVEEAAKTAPGKKRPVEQSPQEPDSSAGIGKSGAQPAKKRLNFGQTGDTESVPDPQPIGEPPAAPSGVGSLTMASGGGAPVADNNEGADGVGSSSGNWHCDSQWLGDRVITTSTRTWALPTYNNHLYKQISNSTSGGSSNDNAYFGYSTPWGYFDFNRFHCHFSPRDWQRLINNNWGFRPKRLNFKLFNIQVKEVTDNNGVKTIANNLTSTVQVFTDSDYQLPYVLGSAHEGCLPPFPADVFMIPQYGYLTLNDGSQAVGRSSFYCLEYFPSQMLRTGNNFQFSYEFENVPFHSSYAHSQSLDRLMNPLIDQYLYYLSRTQSEPRRGDLATIGSQQLLFSQAGPNNMSAQAKNWLPGPCYRQQRVSTTLSQNNNSNFAWTGATKYHLNGRDSLVNPGVAMATHKDDEERFFPSSGVLMFGKQGAGKDNVDYSSVMLTSEEEIKTTNPVATEQYGVVADNLQQQNAAPIVGAVNSQGALPGMVWQNRDVYLQGPIWAKIPHTDGNFHPSPLMGGFGMKHPPPQILIKNTPVPADPPTAFNKDKLNSFITQYSTGQVSVEIEWELQKENSKRWNPEIQYTSNYYKSNNVEFAVNTEGVYSEPRPIGTRYLTRNL

SEQ ID NO: 24 - protein, 742 aa, synthetic construct
  REGION 1..742: note = synthetic polypeptide (Cap9rh74_VR4-5ffo_modified (VP1 protein))
MAADGYLPDWLEDNLSEGIREWWALKPGAPQPKANQQHQDNARGLVLPGYKYLGPGNGLDKGEPVNAADAAALEHDKAYDQQLKAGDNPYLKYNHADAEFQERLKEDTSFGGNLGRAVFQAKKRLLEPLGLVEEAAKTAPGKKRPVEQSPQEPDSSAGIGKSGAQPAKKRLNFGQTGDTESVPDPQPIGEPPAAPSGVGSLTMASGGGAPVADNNEGADGVGSSSGNWHCDSQWLGDRVITTSTRTWALPTYNNHLYKQISNSTSGGSSNDNAYFGYSTPWGYFDFNRFHCHFSPRDWQRLINNNWGFRPKRLNFKLFNIQVKEVTDNNGVKTIANNLTSTVQVFTDSDYQLPYVLGSAHEGCLPPFPADVFMIPQYGYLTLNDGSQAVGRSSFYCLEYFPSQMLRTGNNFQFSYEFENVPFHSSYAHSQSLDRLMNPLIDQYLYYLSRTQSTDQRGDLAELHGQQLLFSQAGPNNMSAQAKNWLPGPCYRQQRVSTTLSQNNNSNFAWTGATKYHLNGRDSLVNPGVAMATHKDDEERFFPSSGVLMFGKQGAGKDNVDYSSVMLTSEEEIKTTNPVATEQYGVVADNLQQQNAAPIVGAVNSQGALPGMVWQNRDVYLQGPIWAKIPHTDGNFHPSPLMGGFGMKHPPPQILIKNTPVPADPPTAFNKDKLNSFITQYSTGQVSVEIEWELQKENSKRWNPEIQYTSNYYKSNNVEFAVNTEGVYSEPRPIGTRYLTRNL

SEQ ID NO: 25 - protein, 742 aa, synthetic construct
  REGION 1..742: note = synthetic polypeptide (Cap9rh74_VR4-5nem (VP1 protein))
MAADGYLPDWLEDNLSEGIREWWALKPGAPQPKANQQHQDNARGLVLPGYKYLGPGNGLDKGEPVNAADAAALEHDKAYDQQLKAGDNPYLKYNHADAEFQERLKEDTSFGGNLGRAVFQAKKRLLEPLGLVEEAAKTAPGKKRPVEQSPQEPDSSAGIGKSGAQPAKKRLNFGQTGDTESVPDPQPIGEPPAAPSGVGSLTMASGGGAPVADNNEGADGVGSSSGNWHCDSQWLGDRVITTSTRTWALPTYNNHLYKQISNSTSGGSSNDNAYFGYSTPWGYFDFNRFHCHFSPRDWQRLINNNWGFRPKRLNFKLFNIQVKEVTDNNGVKTIANNLTSTVQVFTDSDYQLPYVLGSAHEGCLPPFPADVFMIPQYGYLTLNDGSQAVGRSSFYCLEYFPSQMLRTGNNFQFSYEFENVPFHSSYAHSQSLDRLMNPLIDQYLYYLSRTQSAPVRGDLQVLAPQQLLFSQAGPNNMSAQAKNWLPGPCYRQQRVSTTLSQNNNSNFAWTGATKYHLNGRDSLVNPGVAMATHKDDEERFFPSSGVLMFGKQGAGKDNVDYSSVMLTSEEEIKTTNPVATEQYGVVADNLQQQNAAPIVGAVNSQGALPGMVWQNRDVYLQGPIWAKIPHTDGNFHPSPLMGGFGMKHPPPQILIKNTPVPADPPTAFNKDKLNSFITQYSTGQVSVEIEWELQKENSKRWNPEIQYTSNYYKSNNVEFAVNTEGVYSEPRPIGTRYLTRNL

SEQ ID NO: 26 - protein, 742 aa, synthetic construct
  REGION 1..742: note = synthetic polypeptide (Cap9rh74_VR4-5nem_modified (VP1 protein))
MAADGYLPDWLEDNLSEGIREWWALKPGAPQPKANQQHQDNARGLVLPGYKYLGPGNGLDKGEPVNAADAAALEHDKAYDQQLKAGDNPYLKYNHADAEFQERLKEDTSFGGNLGRAVFQAKKRLLEPLGLVEEAAKTAPGKKRPVEQSPQEPDSSAGIGKSGAQPAKKRLNFGQTGDTESVPDPQPIGEPPAAPSGVGSLTMASGGGAPVADNNEGADGVGSSSGNWHCDSQWLGDRVITTSTRTWALPTYNNHLYKQISNSTSGGSSNDNAYFGYSTPWGYFDFNRFHCHFSPRDWQRLINNNWGFRPKRLNFKLFNIQVKEVTDNNGVKTIANNLTSTVQVFTDSDYQLPYVLGSAHEGCLPPFPADVFMIPQYGYLTLNDGSQAVGRSSFYCLEYFPSQMLRTGNNFQFSYEFENVPFHSSYAHSQSLDRLMNPLIDQYLYYLSRTQSAPVRGDLAEINPQQLLFSQAGPNNMSAQAKNWLPGPCYRQQRVSTTLSQNNNSNFAWTGATKYHLNGRDSLVNPGVAMATHKDDEERFFPSSGVLMFGKQGAGKDNVDYSSVMLTSEEEIKTTNPVATEQYGVVADNLQQQNAAPIVGAVNSQGALPGMVWQNRDVYLQGPIWAKIPHTDGNFHPSPLMGGFGMKHPPPQILIKNTPVPADPPTAFNKDKLNSFITQYSTGQVSVEIEWELQKENSKRWNPEIQYTSNYYKSNNVEFAVNTEGVYSEPRPIGTRYLTRNL

SEQ ID NO: 27 - DNA, 2229 bp, synthetic construct
  misc_feature 1..2229: note = synthetic polynucleotide (Cap9rh74_VR4-4um9 (VP1 CDS))
  source 1..2229: mol_type = other DNA
atggctgccgatggttatcttccagattggctcgaggacaaccttagtgaaggaattcgcgagtggtgggctttgaaacctggagcccctcaacccaaggcaaatcaacaacatcaagacaacgctcgaggtcttgtgcttccgggttacaaataccttggacccggcaacggactcgacaagggggagccggtcaacgcagcagacgcggcggccctcgagcacgacaaggcctacgaccagcagctcaaggccggagacaacccgtacctcaagtacaaccacgccgacgccgagttccaggagcggctcaaagaagatacgtcttttgggggcaacctcgggcgagcagtcttccaggccaaaaagaggcttcttgaacctcttggtctggttgaggaagcggctaagacggctcctggaaagaagaggcctgtagagcagtctcctcaggaaccggactcctccgcgggtattggcaaatcgggtgcacagcccgctaaaaagagactcaatttcggtcagactggcgacacagagtcagtcccagaccctcaaccaatcggagaacctcccgcagccccctcaggtgtgggatctcttacaatggcttcaggtggtggcgcaccagtggcagacaataacgaaggtgccgatggagtgggtagttcctcgggaaattggcattgcgattcccaatggctgggggacagagtcatcaccaccagcacccgaacctgggccctgcccacctacaacaatcacctctacaagcaaatctccaacagcacatctggaggatcttcaaatgacaacgcctacttcggctacagcaccccctgggggtattttgacttcaacagattccactgccacttctcaccacgtgactggcagcgactcatcaacaacaactggggattccggcctaagcgactcaacttcaagctcttcaacattcaggtcaaagaggttacggacaacaatggagtcaagaccatcgccaataaccttaccagcacggtccaggtcttcacggactcagactatcagctcccgtacgtgctcgggtcggctcacgagggctgcctcccgccgttcccagcggacgttttcatgattcctcagtacgggtatctgacgcttaatgatggaagccaggccgtgggtcgttcgtccttttactgcctggaatatttcccgtcgcaaatgctaagaacgggtaacaacttccagttcagctacgagtttgagaacgtacctttccatagcagctacgctcacagccaaagcctggaccgactaatgaatccactcatcgaccaatacttgtactatctctcacggactcaaagcaccgacggcagaggcgacctgggcagactgggcccccagcagttgctattttctcaggccgggcctaacaacatgtcggctcaggccaagaactggctacccggtccctgctaccggcagcaacgcgtctccacgacactgtcgcagaacaacaacagcaactttgcctggacgggtgccaccaagtatcatctgaatggcagagactctctggtgaatcctggcgttgccatggctacccacaaggacgacgaagagcgattttttccatccagcggagtcttaatgtttgggaaacagggagctggaaaagacaacgtggactatagcagcgtgatgctaaccagcgaggaagaaataaagaccaccaacccagtggccacagaacagtacggcgtggtggccgataacctgcaacagcaaaacgccgctcctattgtaggggccgtcaatagtcaaggagccttacctggcatggtgtggcagaacagagatgtgtacctgcaaggacccatttgggccaaaattcctcacacggacggcaactttcacccttctccgctgatgggagggtttggaatgaagcacccgcctcctcagatcctcatcaaaaacacacctgtacctgcggatcctccaacggccttcaacaaggacaagctgaactctttcatcacccagtattctactggccaagtcagcgtggagatcgagtgggagctgcagaaggaaaacagcaagcgctggaacccggagatccagtacacttccaactattacaagtctaataatgttgaatttgctgttaatactgaaggtgtatatagtgaaccccgccccattggcaccagtacctgactcgtaatctgtaat

SEQ ID NO: 28 - DNA, 2230 bp, synthetic construct
  misc_feature 1..2230: note = synthetic polynucleotide (Cap9rh74_VR4-4um9_modified (VP1 CDS))
  source 1..2230: mol_type = other DNA
atggctgccgatggttatcttccagattggctcgaggacaaccttagtgaaggaattcgcgagtggtgggctttgaaacctggagcccctcaacccaaggcaaatcaacaacatcaagacaacgctcgaggtcttgtgcttccgggttacaaataccttggacccggcaacggactcgacaagggggagccggtcaacgcagcagacgcggcggccctcgagcacgacaaggcctacgaccagcagctcaaggccggagacaacccgtacctcaagtacaaccacgccgacgccgagttccaggagcggctcaaagaagatacgtcttttgggggcaacctcgggcgagcagtcttccaggccaaaaagaggcttcttgaacctcttggtctggttgaggaagcggctaagacggctcctggaaagaagaggcctgtagagcagtctcctcaggaaccggactcctccgcgggtattggcaaatcgggtgcacagcccgctaaaaagagactcaatttcggtcagactggcgacacagagtcagtcccagaccctcaaccaatcggagaacctcccgcagccccctcaggtgtgggatctcttacaatggcttcaggtggtggcgcaccagtggcagacaataacgaaggtgccgatggagtgggtagttcctcgggaaattggcattgcgattcccaatggctgggggacagagtcatcaccaccagcacccgaacctgggccctgcccacctacaacaatcacctctacaagcaaatctccaacagcacatctggaggatcttcaaatgacaacgcctacttcggctacagcaccccctgggggtattttgacttcaacagattccactgccacttctcaccacgtgactggcagcgactcatcaacaacaactggggattccggcctaagcgactcaacttcaagctcttcaacattcaggtcaaagaggttacggacaacaatggagtcaagaccatcgccaataaccttaccagcacggtccaggtcttcacggactcagactatcagctcccgtacgtgctcgggtcggctcacgagggctgcctcccgccgttcccagcggacgttttcatgattcctcagtacgggtatctgacgcttaatgatggaagccaggccgtgggtcgttcgtccttttactgcctggaatatttcccgtcgcaaatgctaagaacgggtaacaacttccagttcagctacgagtttgagaacgtacctttccatagcagctacgctcacagccaaagcctggaccgactaatgaatccactcatcgaccaatacttgtactatctctcacggactcaaagcagcgagcccagaggcgacctgggcgagctgaacgcccagcagttgctattttctcaggccgggcctaacaacatgtcggctcaggccaagaactggctacccggtccctgctaccggcagcaacgcgtctccacgacactgtcgcagaacaacaacagcaactttgcctggacgggtgccaccaagtatcatctgaatggcagagactctctggtgaatcctggcgttgccatggctacccacaaggacgacgaagagcgattttttccatccagcggagtcttaatgtttgggaaacagggagctggaaaagacaacgtggactatagcagcgtgatgctaaccagcgaggaagaaataaagaccaccaacccagtggccacagaacagtacggcgtggtggccgataacctgcaacagcaaaacgccgctcctattgtaggggccgtcaatagtcaaggagccttacctggcatggtgtggcagaacagagatgtgtacctgcaaggacccatttgggccaaaattcctcacacggacggcaactttcacccttctccgctgatgggagggtttggaatgaagcacccgcctcctcagatcctcatcaaaaacacacctgtacctgcggatcctccaacggccttcaacaaggacaagctgaactctttcatcacccagtattctactggccaagtcagcgtggagatcgagtgggagctgcagaaggaaaacagcaagcgctggaacccggagatccagtacacttccaactattacaagtctaataatgttgaatttgctgttaatactgaaggtgtatatagtgaaccccgccccattggcaccagatacctgactcgtaatctgtaat

SEQ ID NO: 29 - DNA, 2230 bp, synthetic construct
  misc_feature 1..2230: note = synthetic polynucleotide (Cap9rh74_VR4-5ffo (VP1 CDS))
  source 1..2230: mol_type = other DNA
atggctgccgatggttatcttccagattggctcgaggacaaccttagtgaaggaattcgcgagtggtgggctttgaaacctggagcccctcaacccaaggcaaatcaacaacatcaagacaacgctcgaggtcttgtgcttccgggttacaaataccttggacccggcaacggactcgacaagggggagccggtcaacgcagcagacgcggcggccctcgagcacgacaaggcctacgaccagcagctcaaggccggagacaacccgtacctcaagtacaaccacgccgacgccgagttccaggagcggctcaaagaagatacgtcttttgggggcaacctcgggcgagcagtcttccaggccaaaaagaggcttcttgaacctcttggtctggttgaggaagcggctaagacggctcctggaaagaagaggcctgtagagcagtctcctcaggaaccggactcctccgcgggtattggcaaatcgggtgcacagcccgctaaaaagagactcaatttcggtcagactggcgacacagagtcagtcccagaccctcaaccaatcggagaacctcccgcagccccctcaggtgtgggatctcttacaatggcttcaggtggtggcgcaccagtggcagacaataacgaaggtgccgatggagtgggtagttcctcgggaaattggcattgcgattcccaatggctgggggacagagtcatcaccaccagcacccgaacctgggccctgcccacctacaacaatcacctctacaagcaaatctccaacagcacatctggaggatcttcaaatgacaacgcctacttcggctacagcaccccctgggggtattttgacttcaacagattccactgccacttctcaccacgtgactggcagcgactcatcaacaacaactggggattccggcctaagcgactcaacttcaagctcttcaacattcaggtcaaagaggttacggacaacaatggagtcaagaccatcgccaataaccttaccagcacggtccaggtcttcacggactcagactatcagctcccgtacgtgctcgggtcggctcacgagggctgcctcccgccgttcccagcggacgttttcatgattcctcagtacgggtatctgacgcttaatgatggaagccaggccgtgggtcgttcgtccttttactgcctggaatatttcccgtcgcaaatgctaagaacgggtaacaacttccagttcagctacgagtttgagaacgtacctttccatagcagctacgctcacagccaaagcctggaccgactaatgaatccactcatcgaccaatacttgtactatctctcacggactcaaagcgagcccagaagaggcgacctggccaccatcggcagccagcagttgctattttctcaggccgggcctaacaacatgtcggctcaggccaagaactggctacccggtccctgctaccggcagcaacgcgtctccacgacactgtcgcagaacaacaacagcaactttgcctggacgggtgccaccaagtatcatctgaatggcagagactctctggtgaatcctggcgttgccatggctacccacaaggacgacgaagagcgattttttccatccagcggagtcttaatgtttgggaaacagggagctggaaaagacaacgtggactatagcagcgtgatgctaaccagcgaggaagaaataaagaccaccaacccagtggccacagaacagtacggcgtggtggccgataacctgcaacagcaaaacgccgctcctattgtaggggccgtcaatagtcaaggagccttacctggcatggtgtggcagaacagagatgtgtacctgcaaggacccatttgggccaaaattcctcacacggacggcaactttcacccttctccgctgatgggagggtttggaatgaagcacccgcctcctcagatcctcatcaaaaacacacctgtacctgcggatcctccaacggccttcaacaaggacaagctgaactctttcatcacccagtattctactggccaagtcagcgtggagatcgagtgggagctgcagaaggaaaacagcaagcgctggaacccggagatccagtacacttccaactattacaagtctaataatgttgaatttgctgttaatactgaaggtgtatatagtgaaccccgccccattggcaccagatacctgactcgtaatctgtaat

SEQ ID NO: 30 - DNA, 2230 bp, synthetic construct
  misc_feature 1..2230: note = synthetic polynucleotide (Cap9rh74_VR4-5ffo_modified (VP1 CDS))
  source 1..2230: mol_type = other DNA
atggctgccgatggttatcttccagattggctcgaggacaaccttagtgaaggaattcgcgagtggtgggctttgaaacctggagcccctcaacccaaggcaaatcaacaacatcaagacaacgctcgaggtcttgtgcttccgggttacaaataccttggacccggcaacggactcgacaagggggagccggtcaacgcagcagacgcggcggccctcgagcacgacaaggcctacgaccagcagctcaaggccggagacaacccgtacctcaagtacaaccacgccgacgccgagttccaggagcggctcaaagaagatacgtcttttgggggcaacctcgggcgagcagtcttccaggccaaaaagaggcttcttgaacctcttggtctggttgaggaagcggctaagacggctcctggaaagaagaggcctgtagagcagtctcctcaggaaccggactcctccgcgggtattggcaaatcgggtgcacagcccgctaaaaagagactcaatttcggtcagactggcgacacagagtcagtcccagaccctcaaccaatcggagaacctcccgcagccccctcaggtgtgggatctcttacaatggcttcaggtggtggcgcaccagtggcagacaataacgaaggtgccgatggagtgggtagttcctcgggaaattggcattgcgattcccaatggctgggggacagagtcatcaccaccagcacccgaacctgggccctgcccacctacaacaatcacctctacaagcaaatctccaacagcacatctggaggatcttcaaatgacaacgcctacttcggctacagcaccccctgggggtattttgacttcaacagattccactgccacttctcaccacgtgactggcagcgactcatcaacaacaactggggattccggcctaagcgactcaacttcaagctcttcaacattcaggtcaaagaggttacggacaacaatggagtcaagaccatcgccaataaccttaccagcacggtccaggtcttcacggactcagactatcagctcccgtacgtgctcgggtcggctcacgagggctgcctcccgccgttcccagcggacgttttcatgattcctcagtacgggtatctgacgcttaatgatggaagccaggccgtgggtcgttcgtccttttactgcctggaatatttcccgtcgcaaatgctaagaacgggtaacaacttccagttcagctacgagtttgagaacgtacctttccatagcagctacgctcacagccaaagcctggaccgactaatgaatccactcatcgaccaatacttgtactatctctcacggactcaaagcaccgaccagagaggcgacctggccgagctgcacggccagcagttgctattttctcaggccgggcctaacaacatgtcggctcaggccaagaactggctacccggtccctgctaccggcagcaacgcgtctccacgacactgtcgcagaacaacaacagcaactttgcctggacgggtgccaccaagtatcatctgaatggcagagactctctggtgaatcctggcgttgccatggctacccacaaggacgacgaagagcgattttttccatccagcggagtcttaatgtttgggaaacagggagctggaaaagacaacgtggactatagcagcgtgatgctaaccagcgaggaagaaataaagaccaccaacccagtggccacagaacagtacggcgtggtggccgataacctgcaacagcaaaacgccgctcctattgtaggggccgtcaatagtcaaggagccttacctggcatggtgtggcagaacagagatgtgtacctgcaaggacccatttgggccaaaattcctcacacggacggcaactttcacccttctccgctgatgggagggtttggaatgaagcacccgcctcctcagatcctcatcaaaaacacacctgtacctgcggatcctccaacggccttcaacaaggacaagctgaactctttcatcacccagtattctactggccaagtcagcgtggagatcgagtgggagctgcagaaggaaaacagcaagcgctggaacccggagatccagtacacttccaactattacaagtctaataatgttgaatttgctgttaatactgaaggtgtatatagtgaaccccgccccattggcaccagatacctgactcgtaatctgtaat

SEQ ID NO: 31 - DNA, 2230 bp, synthetic construct
  misc_feature 1..2230: note = synthetic polynucleotide (Cap9rh74_VR4-nem (VP1 CDS))
  source 1..2230: mol_type = other DNA
atggctgccgatggttatcttccagattggctcgaggacaaccttagtgaaggaattcgcgagtggtgggctttgaaacctggagcccctcaacccaaggcaaatcaacaacatcaagacaacgctcgaggtcttgtgcttccgggttacaaataccttggacccggcaacggactcgacaagggggagccggtcaacgcagcagacgcggcggccctcgagcacgacaaggcctacgaccagcagctcaaggccggagacaacccgtacctcaagtacaaccacgccgacgccgagttccaggagcggctcaaagaagatacgtcttttgggggcaacctcgggcgagcagtcttccaggccaaaaagaggcttcttgaacctcttggtctggttgaggaagcggctaagacggctcctggaaagaagaggcctgtagagcagtctcctcaggaaccggactcctccgcgggtattggcaaatcgggtgcacagcccgctaaaaagagactcaatttcggtcagactggcgacacagagtcagtcccagaccctcaaccaatcggagaacctcccgcagccccctcaggtgtgggatctcttacaatggcttcaggtggtggcgcaccagtggcagacaataacgaaggtgccgatggagtgggtagttcctcgggaaattggcattgcgattcccaatggctgggggacagagtcatcaccaccagcacccgaacctgggccctgcccacctacaacaatcacctctacaagcaaatctccaacagcacatctggaggatcttcaaatgacaacgcctacttcggctacagcaccccctgggggtattttgacttcaacagattccactgccacttctcaccacgtgactggcagcgactcatcaacaacaactggggattccggcctaagcgactcaacttcaagctcttcaacattcaggtcaaagaggttacggacaacaatggagtcaagaccatcgccaataaccttaccagcacggtccaggtcttcacggactcagactatcagctcccgtacgtgctcgggtcggctcacgagggctgcctcccgccgttcccagcggacgttttcatgattcctcagtacgggtatctgacgcttaatgatggaagccaggccgtgggtcgttcgtccttttactgcctggaatatttcccgtcgcaaatgctaagaacgggtaacaacttccagttcagctacgagtttgagaacgtacctttccatagcagctacgctcacagccaaagcctggaccgactaatgaatccactcatcgaccaatacttgtactatctctcacggactcaaagcgcccccgtgagaggcgacctgcaggtgctggccccccagcagttgctattttctcaggccgggcctaacaacatgtcggctcaggccaagaactggctacccggtccctgctaccggcagcaacgcgtctccacgacactgtcgcagaacaacaacagcaactttgcctggacgggtgccaccaagtatcatctgaatggcagagactctctggtgaatcctggcgttgccatggctacccacaaggacgacgaagagcgattttttccatccagcggagtcttaatgtttgggaaacagggagctggaaaagacaacgtggactatagcagcgtgatgctaaccagcgaggaagaaataaagaccaccaacccagtggccacagaacagtacggcgtggtggccgataacctgcaacagcaaaacgccgctcctattgtaggggccgtcaatagtcaaggagccttacctggcatggtgtggcagaacagagatgtgtacctgcaaggacccatttgggccaaaattcctcacacggacggcaactttcacccttctccgctgatgggagggtttggaatgaagcacccgcctcctcagatcctcatcaaaaacacacctgtacctgcggatcctccaacggccttcaacaaggacaagctgaactctttcatcacccagtattctactggccaagtcagcgtggagatcgagtgggagctgcagaaggaaaacagcaagcgctggaacccggagatccagtacacttccaactattacaagtctaataatgttgaatttgctgttaatactgaaggtgtatatagtgaaccccgccccattggcaccagatacctgactcgtaatctgtaat

SEQ ID NO: 32 - DNA, 2230 bp, synthetic construct; identical to SEQ ID NO: 28
  misc_feature 1..2230: note = synthetic polynucleotide (Cap9rh74_VR4-nem_modified (VP1 CDS))
  source 1..2230: mol_type = other DNA

SEQ ID NO: 33 - protein, 7 aa, synthetic construct
  REGION 1..7: note = synthetic peptide (P1)
RGDLGLS

SEQ ID NO: 34 - protein, 749 aa, synthetic construct
  REGION 1..749: note = synthetic polypeptide (Cap9rh74-HB-P1 (VP1 protein))
MAADGYLPDWLEDNLSEGIREWWALKPGAPQPKANQQHQDNARGLVLPGYKYLGPGNGLDKGEPVNAADAAALEHDKAYDQQLKAGDNPYLKYNHADAEFQERLKEDTSFGGNLGRAVFQAKKRLLEPLGLVEEAAKTAPGKKRPVEQSPQEPDSSAGIGKSGAQPAKKRLNFGQTGDTESVPDPQPIGEPPAAPSGVGSLTMASGGGAPVADNNEGADGVGSSSGNWHCDSQWLGDRVITTSTRTWALPTYNNHLYKQISNSTSGGSSNDNAYFGYSTPWGYFDFNRFHCHFSPRDWQRLINNNWGFRPKRLNFKLFNIQVKEVTDNNGVKTIANNLTSTVQVFTDSDYQLPYVLGSAHEGCLPPFPADVFMIPQYGYLTLNDGSQAVGRSSFYCLEYFPSQMLRTGNNFQFSYEFENVPFHSSYAHSQSLDRLMNPLIDQYLYYLSRTQSTGGTAGTQQLLFSQAGPNNMSAQAKNWLPGPCYRQQRVSTTLSQNNNSNFAWTGATKYHLNGRDSLVNPGVAMATHKDDEERFFPSSGVLMFGKQGAGKDNVDYSSVMLTSEEEIKTTNPVATEQYGVVADNLQQQNAAARGDLGLSSGAAPIVGAVNSQGALPGMVWQNRDVYLQGPIWAKIPHTDGNFHPSPLMGGFGMKHPPPQILIKNTPVPADPPTAFNKDKLNSFITQYSTGQVSVEIEWELQKENSKRWNPEIQYTSNYYKSNNVEFAVNTEGVYSEPRPIGTRYLTRNL

SEQ ID NO: 35 - DNA, 20 bp, synthetic construct
  misc_feature 1..20: note = synthetic oligonucleotide (CMV-FW primer)
  source 1..20: mol_type = other DNA
catcaatgggcgtggatagc

SEQ ID NO: 36 - DNA, 24 bp, synthetic construct
  misc_feature 1..24: note = synthetic oligonucleotide (CMV-RV primer)
  source 1..24: mol_type = other DNA
ggagttgttacgacattttggaaa

SEQ ID NO: 37 - DNA, 18 bp, synthetic construct
  misc_feature 1..18: note = synthetic oligonucleotide (CMV-probe (FAM))
  source 1..18: mol_type = other DNA
atttccaagtctccaccc

SEQ ID NO: 38 - DNA, 20 bp, synthetic construct
  misc_feature 1..20: note = synthetic oligonucleotide (Rplp0-FW primer)
  source 1..20: mol_type = other DNA
ctccaagcagatgcagcaga

SEQ ID NO: 39 - DNA, 20 bp, synthetic construct
  misc_feature 1..20: note = synthetic oligonucleotide (Rplp0-RV primer)
  source 1..20: mol_type = other DNA
atagccttgcgcatcatggt

SEQ ID NO: 40 - DNA, 22 bp, synthetic construct
  misc_feature 1..22: note = synthetic oligonucleotide (Rplp0-probe (VIC))
  source 1..22: mol_type = other DNA
ccgtggtgctgatgggcaagaa

SEQ ID NO: 41 - protein, 7 aa, synthetic construct
  REGION 1..7: note = synthetic peptide (MyoAAV 1A)
RGDLTTP

SEQ ID NO: 42 - protein, 10 aa, synthetic construct
  REGION 1..10: note = synthetic peptide (MyoAAV 2A)
GPGRGDQTTL

SEQ ID NO: 43 - protein, 10 aa, synthetic construct
  REGION 1..10: note = synthetic peptide (MyoAAV 4A)
SNSRGDYNSL

SEQ ID NO: 44 - protein, 10 aa, synthetic construct
  REGION 1..10: note = synthetic peptide (MyoAAV 4E)
ENRRGDFNNT

SEQ ID NO: 45 - protein, 10 aa, synthetic construct
  REGION 1..10: note = synthetic peptide (MyoAAV 3A)
SAQRGDYVGL

SEQ ID NO: 46 - protein, 10 aa, synthetic construct
  REGION 1..10: note = synthetic peptide (MyoAAV 4C)
QERRGDYTSM